European Patent Specification EP 3 703 488 B1, published August 26, 2026. Title: PLANT PROMOTER FOR TRANSGENE EXPRESSION. Applicant: Dow AgroSciences LLC Pioneer Hi-Bred International, Inc. SIDORENKO, LYUDMILA LARSEN, CORY ANTHONY, GENY SREEDHARAN, SRIRAM BUTLER, HOLLY Sims, Lynne Diehn, Scott Rauscher, Gilda Ripp, Kevin Meyer, Knut. The sequence listing filed with the application follows.

SEQUENCE LISTING (29 sequences)

SEQ ID NO: 1 - DNA, 1981 bp, Artificial Sequence
  Synthetic GmCAB2  (promoter/5'UTR and terminator joined by multiple cloning site)
caaattcaaacaaacttacatcccccgaaagctttcaagtaagccgaagtgacctattagcttcgtttttcatgcttccatgattaaaaaagtaattgcagaactccttccagtatatgagctcgaattggggtgccagatatgctaattaattacttttatgatgcaggcaagtgtgttttcagatgctgttcgggatgatgttgatttttataagtatgaactgcactcctttagctttgaagtttgatcactagtggataaattatttatatcttgagctttgaaaatcttccaatgaaacttcattcacactttctgtgaaaaatatcatctattaaagaatcttgtcgtggtcaatgctatgcatgacaacatattaactatttaaaagataacttaaaattataaatagttacatattataaaatgctgtggtggacatgttaccacttgtagaatttatatagtaaaattgaatctataacaacacgacactttatgtttatggaattgtcatgtatgtgataataaataagattaatgaaattattataaaaaacaaggccttaatcgaaaattcaatatctttctatttttttattttataatagtaatataattaaggtgctttattttgttttctcttaattaccgtaattctcatttaaatacaacttttctagcttatgatattgaaagttaattaaaaaaccaataacgtcctgaattttaatctaaaacttctagtacgtttggtttcacattttagatataatttttaaaagttaatagttataaatttgtattttaaatgtgattttttttctatttttaatgactttttaaccatgtacagttattcatactgattttttaaactgtttgcttgaagagaccgtttttgacaccaagttaaagaggtcattatctcttctaaaatcctaagatataatttccaaatgaaaccaaatttgtaatgtagcgaagatgagctgccacattgtgttcttgaggtcgaggcactactagccctgtgtttctgtgtagttttactagcaacacaagttttttctttttttcaaaaataaaaaagaaagaagaaaaaaaatgtgatgggtcactcacgggtttgcaatgttagtgtagcatcagcccaatccaaactatcttccataccaatttccaagttttaatttaaatttaaatttcttgactctgttggacctgaattgtgtggcttacattgaccctctcgaaaacatctgaggaagaagtctttgcatccacgtggcagaataagagccactatagcatgacaaaatatcagcatgagaatccacatccaaatccacgaccaatgaggtgttgctgagttgtgcatatcctcatccacagtatcatacgatcttctataaacctttgtagtagctttcttcattctccacaacacagaacaaaaacaaagaaaaaaaaaaacccttagccaacacaaccatcggatccacacgacaccatggtgagtagttagcttaatcacttaggtcaccgagctcggatgcctacatgcaatgcaatcttctgctcccttttgcagttcccttgtgtttaactccattttcactaatgtaactacacctgtgtagcagaaaaatctgtatgagaaccattatatttttatatattagaaatttgggtccccagaaaatatcaactcttacgtttggaattcaagttaactagttcaaacgttgaaaccatgttcaaggaatctatctattagtgatgtacgtgccttgtacaccatccaattcaaagccatgattaaaaccataaacgaatgaatccatcttccattaccaacaacatccaaagcccacaaggccacaacaagagaaagagcaggcgggcattcaatgtatccatctaaatgcgtcaataatgtagtaagtcataagaaaattaaaaaacaaagaagtga

SEQ ID NO: 2 - DNA, 1299 bp, Artificial Sequence
  Synthetic GmCAB2 promoter
caaattcaaacaaacttacatcccccgaaagctttcaagtaagccgaagtgacctattagcttcgtttttcatgcttccatgattaaaaaagtaattgcagaactccttccagtatatgagctcgaattggggtgccagatatgctaattaattacttttatgatgcaggcaagtgtgttttcagatgctgttcgggatgatgttgatttttataagtatgaactgcactcctttagctttgaagtttgatcactagtggataaattatttatatcttgagctttgaaaatcttccaatgaaacttcattcacactttctgtgaaaaatatcatctattaaagaatcttgtcgtggtcaatgctatgcatgacaacatattaactatttaaaagataacttaaaattataaatagttacatattataaaatgctgtggtggacatgttaccacttgtagaatttatatagtaaaattgaatctataacaacacgacactttatgtttatggaattgtcatgtatgtgataataaataagattaatgaaattattataaaaaacaaggccttaatcgaaaattcaatatctttctatttttttattttataatagtaatataattaaggtgctttattttgttttctcttaattaccgtaattctcatttaaatacaacttttctagcttatgatattgaaagttaattaaaaaaccaataacgtcctgaattttaatctaaaacttctagtacgtttggtttcacattttagatataatttttaaaagttaatagttataaatttgtattttaaatgtgattttttttctatttttaatgactttttaaccatgtacagttattcatactgattttttaaactgtttgcttgaagagaccgtttttgacaccaagttaaagaggtcattatctcttctaaaatcctaagatataatttccaaatgaaaccaaatttgtaatgtagcgaagatgagctgccacattgtgttcttgaggtcgaggcactactagccctgtgtttctgtgtagttttactagcaacacaagttttttctttttttcaaaaataaaaaagaaagaagaaaaaaaatgtgatgggtcactcacgggtttgcaatgttagtgtagcatcagcccaatccaaactatcttccataccaatttccaagttttaatttaaatttaaatttcttgactctgttggacctgaattgtgtggcttacattgaccctctcgaaaacatctgaggaagaagtctttgcatccacgtggcagaa

SEQ ID NO: 3 - DNA, 124 bp, Glycine max
ttgtgcatatcctcatccacagtatcatacgatcttctataaacctttgtagtagctttcttcattctccacaacacagaacaaaaacaaagaaaaaaaaaaacccttagccaacacaaccatc

SEQ ID NO: 4 - DNA, 279 bp, Glycine max
ggatgcctacatgcaatgcaatcttctgctcccttttgcagttcccttgtgtttaactccattttcactaatgtaactacacctgtgtagcagaaaaatctgtatgagaaccattatatttttatatattagaaatttgggtccccagaaaatatcaactcttacgtttggaattcaagttaactagttcaaacgttgaaaccatgttcaaggaatctatctattagtgatgtacgtgccttgtacaccatccaattcaaagccatgattaaaaccata

SEQ ID NO: 5 - DNA, 425 bp, Glycine max
ggatgcctacatgcaatgcaatcttctgctcccttttgcagttcccttgtgtttaactccattttcactaatgtaactacacctgtgtagcagaaaaatctgtatgagaaccattatatttttatatattagaaatttgggtccccagaaaatatcaactcttacgtttggaattcaagttaactagttcaaacgttgaaaccatgttcaaggaatctatctattagtgatgtacgtgccttgtacaccatccaattcaaagccatgattaaaaccataaacgaatgaatccatcttccattaccaacaacatccaaagcccacaaggccacaacaagagaaagagcaggcgggcattcaatgtatccatctaaatgcgtcaataatgtagtaagtcataagaaaattaaaaaacaaagaagtga

SEQ ID NO: 6 - DNA, 1416 bp, Artificial Sequence
  Synthetic GmAct7-2 promoter and 5'UTR from Glyma06g15520
aacaccagtatgacgaggtcgaccaacaatactgggaaacacagccctaggagcatcgtcacagcaaatcctgcctgtacacagatgatcatttaaataaattgagcaataatgaaaccaagactaaatagatgcaattacactaacaagaaactgcaaagtactaaccttcaccattccagttccattgtcacaaacaaggggttgaatatcctcagcatcagccattttttaccaaactacagtacgcatacaataaattgtcagtaccaccaagtttgaatagacaatctacagaacccagccatttacagactttgagggtttacttcaaactctctttttctacacaagacagcatcatagtatatataacacacaaaatcaataggaaagaaaacaaggaaaaaaaataattcagtattatacaatctacttagaaataaaacagtaacaaatgtacataaacagataaaggagccgatcctgtgcattttttaaatgaaactgccaaaattaatagatgaatagaaaacgtccattaggacaccagctaaaatctcagaagtcctctgacacagcatatcttaagttcccaaaccaaatgatcttctactaagaaagatcaatgaggaaaaaaataaagccaaaaaagtgataaaaaaaacagatcagaccataaatccatccaacaccagattatgtaatcgatggctatccacatttcagaataagtaaaggtacagttcaaaaagttcgaagatctctgctatagaagatcggaactgtgatatgtcatttccaccactaaaactacagatcgccacaatctactacatttcattcagtatagatcaggtagtacgaatataaataatcagatacaaaacatccagatatgattttgatgaggtaggtaacaatcttatctcacacagatttaaaaagaaaaacataaaaaagagtactactatggaacaaatctaagaataaacattcgagattgcaaaaagcgctgaatcaaagagcaaaaggaaacgtactttgcatcaaagttatgatgtgagagattaagatgaataccttgtgtgagaagaagaagatggcttagcactcactcacacacacacacactctctctctctccggtgcttgagggctacagaaagaggaaagaggaatgagaagagagaaggggagaaggagagggggtatatatatgcggaaagagagagtgtgtcgttggtgtgagagtgagagtgtaatgtaatgtatttgaaattggaattgaggttgggaccaaaaattgaaattgaaggactggagagagagggaatcatttcgaccacgagaaaagagggatagggtgactggatgacagccttttctttttcatttcacacctttctacccttt

SEQ ID NO: 7 - DNA, 1686 bp, Artificial Sequence
  Synthetic GmGAPC2 promoter and 5' UTR from Glyma0618110
tcaaaccaaggcagcaccctcagtttctgggcgtccagcgagtctggagtgccacatcacacgtggcaacttgaaatcccagggctcagcacggtggagcaaacagcggttgtcccacacaaccacatctccagcagcccattggtgagcatggactctgggagcctggcaggcccagtcaacaagtccttcaaggaagcgctctgattcagctgcatccatgccagggatggcatgggcatggcggccgatcaagaggctgggccttccagtctcaggatgcaccttgaccaatggtctgagaggagttgcagtggtgtccatgccataacctatgtaggctgacccggcctgttggacatgtcccaacttgctctgagaatacacaagggagtgacgagcagacctttggtgaacaagagcacgggttgcctcatcaagggcatcgtaggctgccctcatgtcagcaaagcaggttctgcccccaactgctgggacaacttctgcgctgaacacagctccttgagccatgactggcatgtaggttgagtcggcgtgccaggccatgttgcccacaatgaccttcatcatgtcatcccactcagcaggagagtgctggcgcactgtgccatctgccttgacattggatatggcaacaatgtcacctccgccaatcctctcaattgctccaaagcgtttagcaaaggtaatctgttggtcattgctgaggtgttgcccagggaagatcaagagtgcatgttgaagccaggctgcatggagggcagcgaaaccagcatcgtcaagtgtggcaaggtgaacaccagtgactgtggcacccaaggtggcaccagtgggtgtgatttggagagtggtctgagccatggcagctgccttagctgcggcttcttttgcggcagcctcctttgcagcggcttccttggctgcagcctctttagcggctgcttcctcggcgagattcaacttgtgtccgagcttgctgggaaggtcacagtaacgagcaacagccacctcatgctgttcgacataggtttccttgtctgcctccttgatcctttccaagcgatgatccacatagtagacgccaggcatcttgagattcttagcaggtttctttgagcggtatgtggtcttgaagttgcaaatcaaatggccacctccaaccaacttgagtgccatatcagacctcccctcaagcccaccatcggctgggtaaagcatctcggtgtttgcttcccatccaagggttttcttctgcataactggtccatttgatggaaagttcacacctctaatcttgacattgtagatgagacacccatcttgcaaagaagtgtcttgagtagcggtcaacacgccaccatcttcgtaagttgtaacacgctcccatgtgaaaccctcaggaaaagactgcttaaagaagtcgggaatcccttgtgtgtgattgatgaaagttctggagccatacatgaagctagtggcaagtatgtcgaaggcaaatgggagtggtccaccctcaaccactttgatcctcatggtctgggttccctcataaggcttgccttctccctcggatgtgcatttgaagtgatgattgttgacagtgccctccatgtagagcttcatgtgcatgttctctttgataagttcctcgcctttgctcaccat

SEQ ID NO: 8 - DNA, 632 bp, Glycine max
acaatattcttttcattcatatatcgtgtatccactaggtttgaatgtaaaattattcttgttatctgaaattcttgtgaaattatttactcaactaaaaacataacacgtaacagagcataatcatacacattaataaactcaatactaaaaaatattaaaattaaatttaaccgatagcaaaattagagtatttagatattttcccttcccttggactcctggtaaaccagggatcgtgcaggtatcctcaccattacaacttttaagtgtgtcttcatgcctatagcacactcaaatatcgggcaagtgattcatgaataaactaaaatttgataatttgagtgcgaactgacaatcttatataaaattctcgatacatgtagctatagacattcacattaatgttccgaaggccaaaaaaaatgtgaactctgaaaaaggatacatagaaaataaaataagcattcacaatcactcctttgctacagacaacctactttcgaagacattgatgaattccaaggtgaaaaatgcttctcatcaattctgtgcccgccacatccagagggatgccacacaatatatgatacatcacagctccgaatataccctccaatcctatcccacct

SEQ ID NO: 9 - DNA, 525 bp, Glycine max
cgtttatctagaacttcacggaataatcagtttccaaaaagtactttcacactattacagtataacttatccaaccaattaagttttgaatatcaggtacgccaatcaaaccaatatgaactaaaagccaaaaatgttaatttaaatacggactaaaataagcacagaaaaatgtttaaaccacgaatccaagattcaaagcaaacaggatcaaatatacgagaaccacaaatgaaaaaaaggacggacaaatatctactataacaatcaataacaagtacattagcaagtattcaagccaagtacatcagcgagtatataaaaatccaaaaactcgatccccctccacaagagaaaacatcaaaagtccaaaaaagagctaatgctcctccaacaagtaacaccactggtttcagaaaccgatttattcagacctctcattttttgctcgagcaagacactaaatcgcagctaaacataaacatacggtaataatgtgaagacaagctactttgaagtaacacc

SEQ ID NO: 10 - DNA, 1686 bp, Artificial Sequence
  The coding sequence of the chimeric RFP/AAD12 reporter gene
atggtgagcaaaggcgaggaacttatcaaagagaacatgcacatgaagctctacatggagggcactgtcaacaatcatcacttcaaatgcacatccgagggagaaggcaagccttatgagggaacccagaccatgaggatcaaagtggttgagggtggaccactcccatttgccttcgacatacttgccactagcttcatgtatggctccagaactttcatcaatcacacacaagggattcccgacttctttaagcagtcttttcctgagggtttcacatgggagcgtgttacaacttacgaagatggtggcgtgttgaccgctactcaagacacttctttgcaagatgggtgtctcatctacaatgtcaagattagaggtgtgaactttccatcaaatggaccagttatgcagaagaaaacccttggatgggaagcaaacaccgagatgctttacccagccgatggtgggcttgaggggaggtctgatatggcactcaagttggttggaggtggccatttgatttgcaacttcaagaccacataccgctcaaagaaacctgctaagaatctcaagatgcctggcgtctactatgtggatcatcgcttggaaaggatcaaggaggcagacaaggaaacctatgtcgaacagcatgaggtggctgttgctcgttactgtgaccttcccagcaagctcggacacaagttgaatctcgccgaggaagcagccgctaaagaggctgcagccaaggaagccgctgcaaaggaggctgccgcaaaagaagccgcagctaaggcagctgccatggctcagaccactctccaaatcacacccactggtgccaccttgggtgccacagtcactggtgttcaccttgccacacttgacgatgctggtttcgctgccctccatgcagcctggcttcaacatgcactcttgatcttccctgggcaacacctcagcaatgaccaacagattacctttgctaaacgctttggagcaattgagaggattggcggaggtgacattgttgccatatccaatgtcaaggcagatggcacagtgcgccagcactctcctgctgagtgggatgacatgatgaaggtcattgtgggcaacatggcctggcacgccgactcaacctacatgccagtcatggctcaaggagctgtgttcagcgcagaagttgtcccagcagttgggggcagaacctgctttgctgacatgagggcagcctacgatgcccttgatgaggcaacccgtgctcttgttcaccaaaggtctgctcgtcactcccttgtgtattctcagagcaagttgggacatgtccaacaggccgggtcagcctacataggttatggcatggacaccactgcaactcctctcagaccattggtcaaggtgcatcctgagactggaaggcccagcctcttgatcggccgccatgcccatgccatccctggcatggatgcagctgaatcagagcgcttccttgaaggacttgttgactgggcctgccaggctcccagagtccatgctcaccaatgggctgctggagatgtggttgtgtgggacaaccgctgtttgctccaccgtgctgagccctgggatttcaagttgccacgtgtgatgtggcactccagactcgctggacgcccagaaactgagggtgctgccttggtttga

SEQ ID NO: 11 - DNA, 3661 bp, Artificial Sequence
  Gene expression casette containing the GmCAB2 promoter - GmCAB2 5' UTR - RFP/AAD12 coding sequence - GmCAB2 terminator
caaattcaaacaaacttacatcccccgaaagctttcaagtaagccgaagtgacctattagcttcgtttttcatgcttccatgattaaaaaagtaattgcagaactccttccagtatatgagctcgaattggggtgccagatatgctaattaattacttttatgatgcaggcaagtgtgttttcagatgctgttcgggatgatgttgatttttataagtatgaactgcactcctttagctttgaagtttgatcactagtggataaattatttatatcttgagctttgaaaatcttccaatgaaacttcattcacactttctgtgaaaaatatcatctattaaagaatcttgtcgtggtcaatgctatgcatgacaacatattaactatttaaaagataacttaaaattataaatagttacatattataaaatgctgtggtggacatgttaccacttgtagaatttatatagtaaaattgaatctataacaacacgacactttatgtttatggaattgtcatgtatgtgataataaataagattaatgaaattattataaaaaacaaggccttaatcgaaaattcaatatctttctatttttttattttataatagtaatataattaaggtgctttattttgttttctcttaattaccgtaattctcatttaaatacaacttttctagcttatgatattgaaagttaattaaaaaaccaataacgtcctgaattttaatctaaaacttctagtacgtttggtttcacattttagatataatttttaaaagttaatagttataaatttgtattttaaatgtgattttttttctatttttaatgactttttaaccatgtacagttattcatactgattttttaaactgtttgcttgaagagaccgtttttgacaccaagttaaagaggtcattatctcttctaaaatcctaagatataatttccaaatgaaaccaaatttgtaatgtagcgaagatgagctgccacattgtgttcttgaggtcgaggcactactagccctgtgtttctgtgtagttttactagcaacacaagttttttctttttttcaaaaataaaaaagaaagaagaaaaaaaatgtgatgggtcactcacgggtttgcaatgttagtgtagcatcagcccaatccaaactatcttccataccaatttccaagttttaatttaaatttaaatttcttgactctgttggacctgaattgtgtggcttacattgaccctctcgaaaacatctgaggaagaagtctttgcatccacgtggcagaataagagccactatagcatgacaaaatatcagcatgagaatccacatccaaatccacgaccaatgaggtgttgctgagttgtgcatatcctcatccacagtatcatacgatcttctataaacctttgtagtagctttcttcattctccacaacacagaacaaaaacaaagaaaaaaaaaaacccttagccaacacaaccatcggatccaaacaatggtgagcaaaggcgaggaacttatcaaagagaacatgcacatgaagctctacatggagggcactgtcaacaatcatcacttcaaatgcacatccgagggagaaggcaagccttatgagggaacccagaccatgaggatcaaagtggttgagggtggaccactcccatttgccttcgacatacttgccactagcttcatgtatggctccagaactttcatcaatcacacacaagggattcccgacttctttaagcagtcttttcctgagggtttcacatgggagcgtgttacaacttacgaagatggtggcgtgttgaccgctactcaagacacttctttgcaagatgggtgtctcatctacaatgtcaagattagaggtgtgaactttccatcaaatggaccagttatgcagaagaaaacccttggatgggaagcaaacaccgagatgctttacccagccgatggtgggcttgaggggaggtctgatatggcactcaagttggttggaggtggccatttgatttgcaacttcaagaccacataccgctcaaagaaacctgctaagaatctcaagatgcctggcgtctactatgtggatcatcgcttggaaaggatcaaggaggcagacaaggaaacctatgtcgaacagcatgaggtggctgttgctcgttactgtgaccttcccagcaagctcggacacaagttgaatctcgccgaggaagcagccgctaaagaggctgcagccaaggaagccgctgcaaaggaggctgccgcaaaagaagccgcagctaaggcagctgccatggctcagaccactctccaaatcacacccactggtgccaccttgggtgccacagtcactggtgttcaccttgccacacttgacgatgctggtttcgctgccctccatgcagcctggcttcaacatgcactcttgatcttccctgggcaacacctcagcaatgaccaacagattacctttgctaaacgctttggagcaattgagaggattggcggaggtgacattgttgccatatccaatgtcaaggcagatggcacagtgcgccagcactctcctgctgagtgggatgacatgatgaaggtcattgtgggcaacatggcctggcacgccgactcaacctacatgccagtcatggctcaaggagctgtgttcagcgcagaagttgtcccagcagttgggggcagaacctgctttgctgacatgagggcagcctacgatgcccttgatgaggcaacccgtgctcttgttcaccaaaggtctgctcgtcactcccttgtgtattctcagagcaagttgggacatgtccaacaggccgggtcagcctacataggttatggcatggacaccactgcaactcctctcagaccattggtcaaggtgcatcctgagactggaaggcccagcctcttgatcggccgccatgcccatgccatccctggcatggatgcagctgaatcagagcgcttccttgaaggacttgttgactgggcctgccaggctcccagagtccatgctcaccaatgggctgctggagatgtggttgtgtgggacaaccgctgtttgctccaccgtgctgagccctgggatttcaagttgccacgtgtgatgtggcactccagactcgctggacgcccagaaactgagggtgctgccttggtttgagtagttagcttaatcacctagagctcggtcaccgagctcggatgcctacatgcaatgcaatcttctgctcccttttgcagttcccttgtgtttaactccattttcactaatgtaactacacctgtgtagcagaaaaatctgtatgagaaccattatatttttatatattagaaatttgggtccccagaaaatatcaactcttacgtttggaattcaagttaactagttcaaacgttgaaaccatgttcaaggaatctatctattagtgatgtacgtgccttgtacaccatccaattcaaagccatgattaaaaccataaacgaatgaatccatcttccattaccaacaacatccaaagcccacaaggccacaacaagagaaagagcaggcgggcattcaatgtatccatctaaatgcgtcaataatgtagtaagtcataagaaaattaaaaaacaaagaagtga

SEQ ID NO: 12 - DNA, 4584 bp, Artificial Sequence
  Gene expression cassette containing the GFP and PAT reporter/selectable marker genes
gtcgacctgcaggtcaacggatcaggatattcttgtttaagatgttgaactctatggaggtttgtatgaactgatgatctaggaccggataagttcccttcttcatagcgaacttattcaaagaatgttttgtgtatcattcttgttacattgttattaatgaaaaaatattattggtcattggactgaacacgagtgttaaatatggaccaggccccaaataagatccattgatatatgaattaaataacaagaataaatcgagtcaccaaaccacttgccttttttaacgagacttgttcaccaacttgatacaaaagtcattatcctatgcaaatcaataatcatacaaaaatatccaataacactaaaaaattaaaagaaatggataatttcacaatatgttatacgataaagaagttacttttccaagaaattcactgattttataagcccacttgcattagataaatggcaaaaaaaaacaaaaaggaaaagaaataaagcacgaagaattctagaaaatacgaaatacgcttcaatgcagtgggacccacggttcaattattgccaattttcagctccaccgtatatttaaaaaataaaacgataatgctaaaaaaatataaatcgtaacgatcgttaaatctcaacggctggatcttatgacgaccgttagaaattgtggttgtcgacgagtcagtaataaacggcgtcaaagtggttgcagccggcacacacgagtcgtgtttatcaactcaaagcacaaatacttttcctcaacctaaaaataaggcaattagccaaaaacaactttgcgtgtaaacaacgctcaatacacgtgtcattttattattagctattgcttcaccgccttagctttctcgtgacctagtcgtcctcgtcttttcttcttcttcttctataaaacaatacccaaagcttcttcttcacaattcagatttcaatttctcaaaatcttaaaaactttctctcaattctctctaccgtgatcaaggtaaatttctgtgttccttattctctcaaaatcttcgattttgttttcgttcgatcccaatttcgtatatgttctttggtttagattctgttaatcttagatcgaagacgattttctgggtttgatcgttagatatcatcttaattctcgattagggtttcataaatatcatccgatttgttcaaataatttgagttttgtcgaataattactcttcgatttgtgatttctatctagatctggtgttagtttctagtttgtgcgatcgaatttgtcgattaatctgagtttttctgattaacagagatctccatggctcctgccatgaagattgaatgccgcatcactggcaccctcaacggtgtggagtttgaattggttggaggtggagagggcacacctgaacaagggaggatgaccaacaagatgaagtcaactaaaggggctctcaccttcagcccatacttgctttctcatgtcatgggctatggattctaccactttggcacctacccctctggatatgagaaccctttccttcatgccatcaacaatggaggctacacaaacaccagaattgagaagtacgaagatggtggagtcttgcatgtctccttcagctaccgctatgaggctgggagggtcataggagacttcaaagttgtgggcactggattcccagaggactcagtcatcttcactgacaagatcataaggagcaatgccactgttgagcacctccatccaatgggtgacaatgtgcttgttggttcatttgcacgtaccttcagcctcagagatggtggctactattcctttgtggttgattctcacatgcacttcaaatctgcaatccacccctccatcctccagaatgggggtccaatgtttgctttcagacgtgtggaagagttgcacagcaacacagaacttggcattgtggagtaccagcatgccttcaagacacccattgcatttgcttgagtagttagcttaatcacttaggtcaccagcataatttttattaatgtactaaattactgttttgttaaatgcaattttgctttctcgggattttaatatcaaaatctatttagaaatacacaatattttgttgcaggcttgctggagaatcgatctgctatcataaaaattacaaaaaaattttatttgcctcaattattttaggattggtattaaggacgcttaaattatttgtcgggtcactacgcatcattgtgattgagaagatcagcgatacgaaatattcgtagtactatcgataatttatttgaaaattcataagaaaagcaaacgttacatgaattgatgaaacaatacaaagacagataaagccacgcacatttaggatattggccgagattactgaatattgagtaagatcacggaatttctgacaggagcatgtcttcaattcagcccaaatggcagttgaaatactcaaaccgccccatatgcaggagcggatcattcattgtttgtttggttgcctttgccaacatgggagtccaaggttgcggccgcttaattaacttactagtgctagcctcgaggtcgactctgatcatggatgctacgtcacggcagtacaggactatcatcttgaaagtcgattgagcatcgaaacccagctttcttgtacaaagtggttgcggccgcttaattaaatttaaatgtttgggaagctaggccaccgtggcccgcctgcaggggaagcttgtttaaacccagaaggtaattatccaagatgtagcatcaagaatccaatgtttacgggaaaaactatggaagtattatgtaagctcagcaagaagcagatcaatatgcggcacatatgcaacctatgttcaaaaatgaagaatgtacagatacaagatcctatactgccagaatacgaagaagaatacgtagaaattgaaaaagaagaaccaggcgaagaaaagaatcttgaagacgtaagcactgacgacaacaatgaaaagaagaagataaggtcggtgattgtgaaagagacatagaggacacatgtaaggtggaaaatgtaagggcggaaagtaaccttatcacaaaggaatcttatcccccactacttatccttttatatttttccgtgtcatttttgcccttgagttttcctatataaggaaccaagttcggcatttgtgaaaacaagaaaaaatttggtgtaagctattttctttgaagtactgaggatacaacttcagagaaatttgtaagtttgtagatctccatgtctccggagaggagaccagttgagattaggccagctacagcagctgatatggccgcggtttgtgatatcgttaaccattacattgagacgtctacagtgaactttaggacagagccacaaacaccacaagagtggattgatgatctagagaggttgcaagatagatacccttggttggttgctgaggttgagggtgttgtggctggtattgcttacgctgggccctggaaggctaggaacgcttacgattggacagttgagagtactgtttacgtgtcacataggcatcaaaggttgggcctaggatccacattgtacacacatttgcttaagtctatggaggcgcaaggttttaagtctgtggttgctgttataggccttccaaacgatccatctgttaggttgcatgaggctttgggatacacagcccgtggtacattgcgcgcagctggatacaagcatggtggatggcatgatgttggtttttggcaaagggattttgagttgccagctcctccaaggccagttaggccagttacccagatctgactgagcttgagcttatgagcttatgagcttagagctcagatcggcggcaatagcttcttagcgccatcccgggttgatcctatctgtgttgaaatagttgcggtgggcaaggctctctttcagaaagacaggcggccaaaggaacccaaggtgaggtgggctatggctctcagttccttgtggaagcgcttggtctaaggtgcagaggtgttagcggggatgaagcaaaagtgtccgattgtaacaagatatgttgatcctacgtaaggatattaaagtatgtattcatcactaatataatcagtgtattccaatatgtactacgatttccaatgtctttattgtcgccgtatgcaatcggcgtcacaaaataatccccggtgactttcttttaatccaggatgaaataatatgttattataatttttgcgatttggtccgttataggaattgaagtgtgcttgcggtcgccaccactcccatttcataattttacatgtatttgaaaaataaaaatttatggtattcaatttaaacacgtatacttgtaaagaatgatatcttgaaagaaatatagtttaaatatttattgataaaataacaagtcaggtattatagtccaagcaaaaacataaatttattgatgcaagtttaaattcagaaatatttcaataactgattatatcagctggtacattgccgtagatgaaagactgagtgcgatattatggtgtaatacata

SEQ ID NO: 13 - DNA, 22 bp, artificial sequence
  Primer sequence
gaggattagggtttcaacggag

SEQ ID NO: 14 - DNA, 21 bp, Artificial Sequence
  Primer Sequence
gagaattgagctgagacgagg

SEQ ID NO: 15 - DNA, 25 bp, Artificial Sequence
  Probe Sequence
agagaagtttcgacggatttcgggc

SEQ ID NO: 16 - DNA, 29 bp, Artificial Sequence
  Primer Sequence
acaagagtggattgatgatctagagaggt

SEQ ID NO: 17 - DNA, 29 bp, Artificial Sequence
  Primer Sequence
ctttgatgcctatgtgacacgtaaacagt

SEQ ID NO: 18 - DNA, 29 bp, Artificial Sequence
  Probe Sequence
agggtgttgtggctggtattgcttacgct

SEQ ID NO: 19 - DNA, 20 bp, Artificial Sequence
  Primer Sequence
cagagtccatgctcaccaat

SEQ ID NO: 20 - DNA, 19 bp, Artificial Sequence
  Primer Sequence
acgtggcaacttgaaatcc

SEQ ID NO: 21 - DNA, 24 bp, Artificial Sequence
  Probe Sequence
tggagatgtggttgtgtgggacaa

SEQ ID NO: 22 - DNA, 26 bp, artificial sequence
  Primer Sequence
acaagagtggattgatgatctagaga

SEQ ID NO: 23 - DNA, 26 bp, Artificial Sequence
  Primer Sequence
ctttgatgcctatgtgacacgtaaac

SEQ ID NO: 24 - DNA, 29 bp, Artificial Sequence
  Probe Sequence
ccagcgtaagcaataccagccacaacacc

SEQ ID NO: 25 - DNA, 21 bp, Artificial Sequence
  Primer Sequence
cgccgaagtatcgactcaact

SEQ ID NO: 26 - DNA, 19 bp, Artificial Sequence
  Primer Sequence
gcaacgtcggttcgagatg

SEQ ID NO: 27 - DNA, 24 bp, Artificial Sequence
  Probe Sequence
tcagaggtagttggcgtcatcgag

SEQ ID NO: 28 - DNA, 1453 bp, Glycine max
gcagatgaagataaagaaaatgaaaagataaactaaattagtctagactttcttggctaaagtagagctttagagtacaaattcaaacaaacttacatcccccgaaagtcttcaagtaagccgaagtgacctattagcttcgtttttcatgcttccatgattaaaaaagtaattgcagaactccttccagtatatgagctcgaattggggtgccagatatgctaattaattacttttatgatgcaggcaagtgtgttttcagatgctgttcgggatgatgttgatttttataagtatgaactgcactcctttagctttgaagtttgatcactagtggataaattatttatatcttgagctttgaaaatcttccaatgaaacttcattcacactttctgtgaaaaatatcatctattaaagaatcttgtcgtggtcaatgctatgcatgacaacatattaactatttaaaagataacttaaaattataaatagttacatattataaaatgctgtggtggacatgttaccacttgtagaatttatatagtaaaattgaatctataacaacacgacactttatgtttatggaattgtcatgtatgtgataataaataagattaatgaaattattataaaaaacaaggccttaatcgaaaattcaatatctttctatttttttattttataatagtaatataattaaggtgctttattttgttttctcttaattaccgtaattctcatttaaatacaacttttctagcttatgatattgaaagttaattaaaaaaccaataacgtcctgaattttaatctaaaacttctagtacgtttggtttcacattttagatataatttttaaaagttaatagttataaatttgtattttaaatgtgattttttttctatttttaatgactttttaaccatgtacagttattcatactgattttttaaactgtttgcttgaagagaccgtttttgacaccaagttaaagaggtcattatctcttctaaaatcctaagatataatttccaaatgaaaccaaatttgtaatgtagcgaagatgagctgccacattgtgttcttgaggtcgaggcactactagccctgtgtttctgtgtagttttactagcaacacaagttttttctttttttcaaaaataaaaaagaaagaagaaaaaaaatgtgatgggtcactcacgggtttgcaatgttagtgtagcatcagcccaatccaaactatcttccataccaatttccaagttttaatttaaatttaaatttcttgactctgttggacctgaattgtgtggcttacattgaccctctcgaaaacatctgaggaagaagtctttgcatccacgtggcagaataagagccactatagcatgacaaaatatcagcatgagaatccacatccaaatccacgaccaatgaggtgttgctgag

SEQ ID NO: 29 - DNA, 1454 bp, Glycine max
agcagatgaagataaagaaaatgaaaagataaactaaattagtctagactttcttggctaaagtagagctttagagtacaaattcaaacaaacttacatcccccgaaagtcttcaagtaagccgaagtgacctattagcttcgtttttcatgcttccatgattaaaaaagtaattgcagaactccttccagtatatgagctcgaattggggtgccagatatgctaattaattacttttatgatgcaggcaagtgtgttttcagatgctgttcgggatgatgttgatttttataagtatgaactgcactcctttagctttgaagtttgatcactagtggataaattatttatatcttgagctttgaaaatcttccaatgaaacttcattcacactttctgtgaaaaatatcatctattaaagaatcttgtcgtggtcaatgctatgcatgacaacatattaactatttaaaagataacttaaaattataaatagttacatattataaaatgctgtggtggacatgttaccacttgtagaatttatatagtaaaattgaatctataacaacacgacactttatgtttatggaattgtcatgtatgtgataataaataagattaatgaaattattataaaaaacaaggccttaatcgaaaattcaatatctttctatttttttattttataatagtaatataattaaggtgctttattttgttttctcttaattaccgtaattctcatttaaatacaacttttctagcttatgatattgaaagttaattaaaaaaccaataacgtcctgaattttaatctaaaacttctagtacgtttggtttcacattttagatataatttttaaaagttaatagttataaatttgtattttaaatgtgattttttttctatttttaatgactttttaaccatgtacagttattcatactgattttttaaactgtttgcttgaagagaccgtttttgacaccaagttaaagaggtcattatctcttctaaaatcctaagatataatttccaaatgaaaccaaatttgtaatgtagcgaagatgagctgccacattgtgttcttgaggtcgaggcactactagccctgtgtttctgtgtagttttactagcaacacaagttttttctttttttcaaaaataaaaaagaaagaagaaaaaaaatgtgatgggtcactcacgggtttgcaatgttagtgtagcatcagcccaatccaaactatcttccataccaatttccaagttttaatttaaatttaaatttcttgactctgttggacctgaattgtgtggcttacattgaccctctcgaaaacatctgaggaagaagtctttgcatccacgtggcagaataagagccactatagcatgacaaaatatcagcatgagaatccacatccaaatccacgaccaatgaggtgttgctgag